European Patent Application EP 4 549 465 A1, published May 7, 2025. Title: MUTANT OF ANTIBODY VARIABLE REGION AND USE THEREOF. Applicant: SHENYANG PHARMACEUTICAL UNIVERSITY. The sequence listing filed with the application follows.

SEQUENCE LISTING (133 sequences)

SEQ ID NO: 1 - DNA, 360 bp, synthetic construct
  source 1..360: mol_type = other DNA
gaagtgcagctggtggaatccggaggaggactggtgcaacctggagggtccctgaggttgtcttgtgctgcctccggcttcaacatcaaggacacctacatccactgggtgaggcaagctcctggcaaaggactggaatgggtggctaggatctatcccaccaacggctacacaaggtatgccgactccgtgaagggaaggttcaccatctctgccgacacctccaagaataccgcctacctgcagatgaattccctgagggccgaagacacagctgtgtactactgctccaggtggggcggagatggcttttacgccatggactactggggacagggaacactggtgaccgtttcctcc

SEQ ID NO: 2 - DNA, 321 bp, synthetic construct
  source 1..321: mol_type = other DNA
gatatccagatgacccagtccccttcttccctgtccgcttctgtgggagacagggtgacaatcacctgtagggcctcccaggacgtgaatacagctgtggcctggtaccaacaaaagcccggcaaagctcccaaactgctgatttactccgcctccttcctgtattctggagtgccctccaggttttctgggtccaggtccggaacagacttcacactgaccatctcctccctgcagcctgaagacttcgccacctactactgccagcagcactataccaccccccctacatttggacaaggcaccaaggtggagattaag

SEQ ID NO: 3 - DNA, 45 bp, synthetic construct
  source 1..45: mol_type = other DNA
ggaggaggaggatctggaggaggaggatctggaggaggaggaagc

SEQ ID NO: 4 - protein, 120 aa, synthetic construct [sequence omitted]

SEQ ID NO: 5 - protein, 107 aa, synthetic construct [sequence omitted]

SEQ ID NO: 6 - protein, 15 aa, synthetic construct
GGGGSGGGGSGGGGS

SEQ ID NO: 7 - DNA, 360 bp, synthetic construct
  source 1..360: mol_type = other DNA
gaagtgcagctggtggaatccggaggaggactgtgtcaacctggagggtccctgaggttgtcttgtgctgcctccggcttcaacatcaaggacacctacatccactgggtgaggcaagctcctggcaaaggactggaatgggtggctaggatctatcccaccaacggctacacaaggtatgccgactccgtgaagggaaggttcaccatctctgccgacacctccaagaataccgcctacctgcagatgaattccctgagggccgaagacacagctgtgtactactgctccaggtggggcggagatggcttttacgccatggactactggggacagggaacactggtgaccgtttcctcc

SEQ ID NO: 8 - protein, 120 aa, synthetic construct
EVQLVESGGGLCQPGGSLRLSCAASGFNIKDTYIHWVRQAPGKGLEWVARIYPTNGYTRYADSVKGRFTISADTSKNTAYLQMNSLRAEDTAVYYCSRWGGDGFYAMDYWGQGTLVTVSS

SEQ ID NO: 9 - DNA, 360 bp, synthetic construct
  source 1..360: mol_type = other DNA
gaagtgcagctggtggaatccggaggaggactggtgcaacctggagggtccctgaggttgtcttgtgctgcctccggcttcaacatcaaggacacctacatctgttgggtgaggcaagctcctggcaaaggactggaatgggtggctaggatctatcccaccaacggctacacaaggtatgccgactccgtgaagggaaggttcaccatctctgccgacacctccaagaataccgcctacctgcagatgaattccctgagggccgaagacacagctgtgtactactgctccaggtggggcggagatggcttttacgccatggactactggggacagggaacactggtgaccgtttcctcc

SEQ ID NO: 10 - protein, 120 aa, synthetic construct
EVQLVESGGGLVQPGGSLRLSCAASGFNIKDTYICWVRQAPGKGLEWVARIYPTNGYTRYADSVKGRFTISADTSKNTAYLQMNSLRAEDTAVYYCSRWGGDGFYAMDYWGQGTLVTVSS

SEQ ID NO: 11 - DNA, 360 bp, synthetic construct
  source 1..360: mol_type = other DNA
gaagtgcagctggtggaatccggaggaggactggtgcaacctggagggtccctgaggttgtcttgtgctgcctccggcttcaacatcaaggacacctacatccactgggtgaggcaagctcctggcaaaggactggaatgggtggctaggatctatcccaccaacggctacacaaggtattgtgactccgtgaagggaaggttcaccatctctgccgacacctccaagaataccgcctacctgcagatgaattccctgagggccgaagacacagctgtgtactactgctccaggtggggcggagatggcttttacgccatggactactggggacagggaacactggtgaccgtttcctcc

SEQ ID NO: 12 - protein, 120 aa, synthetic construct
EVQLVESGGGLVQPGGSLRLSCAASGFNIKDTYIHWVRQAPGKGLEWVARIYPTNGYTRYCDSVKGRFTISADTSKNTAYLQMNSLRAEDTAVYYCSRWGGDGFYAMDYWGQGTLVTVSS

SEQ ID NO: 13 - DNA, 321 bp, synthetic construct
  source 1..321: mol_type = other DNA
gatatccagatgacccagtccccttcttccctgtccgcttctgtgggagacagggtgacatgtacctgtagggcctcccaggacgtgaatacagctgtggcctggtaccaacaaaagcccggcaaagctcccaaactgctgatttactccgcctccttcctgtattctggagtgccctccaggttttctgggtccaggtccggaacagacttcacactgaccatctcctccctgcagcctgaagacttcgccacctactactgccagcagcactataccaccccccctacatttggacaaggcaccaaggtggagattaag

SEQ ID NO: 14 - protein, 107 aa, synthetic construct
DIQMTQSPSSLSASVGDRVTCTCRASQDVNTAVAWYQQKPGKAPKLLIYSASFLYSGVPSRFSGSRSGTDFTLTISSLQPEDFATYYCQQHYTTPPTFGQGTKVEIK

SEQ ID NO: 15 - DNA, 321 bp, synthetic construct
  source 1..321: mol_type = other DNA
gatatccagatgacccagtccccttcttccctgtccgcttctgtgggagacagggtgacaatcacctgtagggcctcccaggacgtgaatacagctgtggcctggtaccaacaaaagcccggcaaagctcccaaactgtgtatttactccgcctccttcctgtattctggagtgccctccaggttttctgggtccaggtccggaacagacttcacactgaccatctcctccctgcagcctgaagacttcgccacctactactgccagcagcactataccaccccccctacatttggacaaggcaccaaggtggagattaag

SEQ ID NO: 16 - protein, 107 aa, synthetic construct
DIQMTQSPSSLSASVGDRVTITCRASQDVNTAVAWYQQKPGKAPKLCIYSASFLYSGVPSRFSGSRSGTDFTLTISSLQPEDFATYYCQQHYTTPPTFGQGTKVEIK

SEQ ID NO: 17 - DNA, 321 bp, synthetic construct
  source 1..321: mol_type = other DNA
gatatccagatgacccagtccccttcttccctgtccgcttctgtgggagacagggtgacaatcacctgtagggcctcccaggacgtgaatacagctgtggcctggtaccaacaaaagcccggcaaagctcccaaactgctgtgttactccgcctccttcctgtattctggagtgccctccaggttttctgggtccaggtccggaacagacttcacactgaccatctcctccctgcagcctgaagacttcgccacctactactgccagcagcactataccaccccccctacatttggacaaggcaccaaggtggagattaag

SEQ ID NO: 18 - protein, 107 aa, synthetic construct
DIQMTQSPSSLSASVGDRVTITCRASQDVNTAVAWYQQKPGKAPKLLCYSASFLYSGVPSRFSGSRSGTDFTLTISSLQPEDFATYYCQQHYTTPPTFGQGTKVEIK

SEQ ID NO: 19 - DNA, 321 bp, synthetic construct
  source 1..321: mol_type = other DNA
gatatccagatgacccagtccccttcttccctgtccgcttctgtgggagacagggtgacaatcacctgtagggcctcccaggacgtgaatacagctgtggcctggtaccaacaaaagcccggcaaagctcccaaactgctgatttactccgcctccttcctgtattctggagtgccctccaggttttctgggtccaggtccggaacagactgtacactgaccatctcctccctgcagcctgaagacttcgccacctactactgccagcagcactataccaccccccctacatttggacaaggcaccaaggtggagattaag

SEQ ID NO: 20 - protein, 107 aa, synthetic construct
DIQMTQSPSSLSASVGDRVTITCRASQDVNTAVAWYQQKPGKAPKLLIYSASFLYSGVPSRFSGSRSGTDCTLTISSLQPEDFATYYCQQHYTTPPTFGQGTKVEIK

SEQ ID NO: 21 - DNA, 321 bp, synthetic construct
  source 1..321: mol_type = other DNA
gatatccagatgacccagtccccttcttccctgtccgcttctgtgggagacagggtgacaatcacctgtagggcctcccaggacgtgaatacagctgtggcctggtaccaacaaaagcccggcaaagctcccaaactgctgatttactccgcctccttcctgtattctggagtgccctccaggttttctgggtccaggtccggaacagacttcacactgacctgttcctccctgcagcctgaagacttcgccacctactactgccagcagcactataccaccccccctacatttggacaaggcaccaaggtggagattaag

SEQ ID NO: 22 - protein, 107 aa, synthetic construct
DIQMTQSPSSLSASVGDRVTITCRASQDVNTAVAWYQQKPGKAPKLLIYSASFLYSGVPSRFSGSRSGTDFTLTCSSLQPEDFATYYCQQHYTTPPTFGQGTKVEIK

SEQ ID NO: 23 - DNA, 360 bp, synthetic construct
  source 1..360: mol_type = other DNA
gaagtgcagctggtggaatccggaggaggactggtgcaacctggagggtccctgaggttgtcttgtgctgcctccggcttcaacatcaaggacacctactgtcactgggtgaggcaagctcctggcaaaggactggaatgggtggctaggatctatcccaccaacggctacacaaggtatgccgactccgtgaagggaaggttcaccatctctgccgacacctccaagaataccgcctacctgcagatgaattccctgagggccgaagacacagctgtgtactactgctccaggtggggcggagatggcttttacgccatggactactggggacagggaacactggtgaccgtttcctcc

SEQ ID NO: 24 - protein, 120 aa, synthetic construct
EVQLVESGGGLVQPGGSLRLSCAASGFNIKDTYCHWVRQAPGKGLEWVARIYPTNGYTRYADSVKGRFTISADTSKNTAYLQMNSLRAEDTAVYYCSRWGGDGFYAMDYWGQGTLVTVSS

SEQ ID NO: 25 - DNA, 360 bp, synthetic construct
  source 1..360: mol_type = other DNA
gaagtgcagctggtggaatccggaggaggactggtgcaacctggagggtccctgaggttgtcttgtgctgcctccggcttcaacatcaaggacacctacatccactgggtgtgtcaagctcctggcaaaggactggaatgggtggctaggatctatcccaccaacggctacacaaggtatgccgactccgtgaagggaaggttcaccatctctgccgacacctccaagaataccgcctacctgcagatgaattccctgagggccgaagacacagctgtgtactactgctccaggtggggcggagatggcttttacgccatggactactggggacagggaacactggtgaccgtttcctcc

SEQ ID NO: 26 - protein, 120 aa, synthetic construct
EVQLVESGGGLVQPGGSLRLSCAASGFNIKDTYIHWVCQAPGKGLEWVARIYPTNGYTRYADSVKGRFTISADTSKNTAYLQMNSLRAEDTAVYYCSRWGGDGFYAMDYWGQGTLVTVSS

SEQ ID NO: 27 - DNA, 360 bp, synthetic construct
  source 1..360: mol_type = other DNA
gaagtgcagctggtggaatccggaggaggactggtgcaacctggagggtccctgaggttgtcttgtgctgcctccggcttcaacatcaaggacacctacatccactgggtgaggcaagctcctggcaaatgtctggaatgggtggctaggatctatcccaccaacggctacacaaggtatgccgactccgtgaagggaaggttcaccatctctgccgacacctccaagaataccgcctacctgcagatgaattccctgagggccgaagacacagctgtgtactactgctccaggtggggcggagatggcttttacgccatggactactggggacagggaacactggtgaccgtttcctcc

SEQ ID NO: 28 - protein, 120 aa, synthetic construct
EVQLVESGGGLVQPGGSLRLSCAASGFNIKDTYIHWVRQAPGKCLEWVARIYPTNGYTRYADSVKGRFTISADTSKNTAYLQMNSLRAEDTAVYYCSRWGGDGFYAMDYWGQGTLVTVSS

SEQ ID NO: 29 - DNA, 360 bp, synthetic construct
  source 1..360: mol_type = other DNA
gaagtgcagctggtggaatccggaggaggactggtgcaacctggagggtccctgaggttgtcttgtgctgcctccggcttcaacatcaaggacacctacatccactgggtgaggcaagctcctggcaaaggactggaatgtgtggctaggatctatcccaccaacggctacacaaggtatgccgactccgtgaagggaaggttcaccatctctgccgacacctccaagaataccgcctacctgcagatgaattccctgagggccgaagacacagctgtgtactactgctccaggtggggcggagatggcttttacgccatggactactggggacagggaacactggtgaccgtttcctcc

SEQ ID NO: 30 - protein, 120 aa, synthetic construct
EVQLVESGGGLVQPGGSLRLSCAASGFNIKDTYIHWVRQAPGKGLECVARIYPTNGYTRYADSVKGRFTISADTSKNTAYLQMNSLRAEDTAVYYCSRWGGDGFYAMDYWGQGTLVTVSS

SEQ ID NO: 31 - DNA, 360 bp, synthetic construct
  source 1..360: mol_type = other DNA
gaagtgcagctggtggaatccggaggaggactggtgcaacctggagggtccctgaggttgtcttgtgctgcctccggcttcaacatcaaggacacctacatccactgggtgaggcaagctcctggcaaaggactggaatgggtggctaggtgttatcccaccaacggctacacaaggtatgccgactccgtgaagggaaggttcaccatctctgccgacacctccaagaataccgcctacctgcagatgaattccctgagggccgaagacacagctgtgtactactgctccaggtggggcggagatggcttttacgccatggactactggggacagggaacactggtgaccgtttcctcc

SEQ ID NO: 32 - protein, 120 aa, synthetic construct
EVQLVESGGGLVQPGGSLRLSCAASGFNIKDTYIHWVRQAPGKGLEWVARCYPTNGYTRYADSVKGRFTISADTSKNTAYLQMNSLRAEDTAVYYCSRWGGDGFYAMDYWGQGTLVTVSS

SEQ ID NO: 33 - DNA, 360 bp, synthetic construct
  source 1..360: mol_type = other DNA
gaagtgcagctggtggaatccggaggaggactggtgcaacctggagggtccctgaggttgtcttgtgctgcctccggcttcaacatcaaggacacctacatccactgggtgaggcaagctcctggcaaaggactggaatgggtggctaggatctatcccaccaacggctacacaaggtgtgccgactccgtgaagggaaggttcaccatctctgccgacacctccaagaataccgcctacctgcagatgaattccctgagggccgaagacacagctgtgtactactgctccaggtggggcggagatggcttttacgccatggactactggggacagggaacactggtgaccgtttcctcc

SEQ ID NO: 34 - protein, 120 aa, synthetic construct
EVQLVESGGGLVQPGGSLRLSCAASGFNIKDTYIHWVRQAPGKGLEWVARIYPTNGYTRCADSVKGRFTISADTSKNTAYLQMNSLRAEDTAVYYCSRWGGDGFYAMDYWGQGTLVTVSS

SEQ ID NO: 35 - DNA, 360 bp, synthetic construct
  source 1..360: mol_type = other DNA
gaagtgcagctggtggaatccggaggaggactggtgcaacctggagggtccctgaggttgtcttgtgctgcctccggcttcaacatcaaggacacctacatccactgggtgaggcaagctcctggcaaaggactggaatgggtggctaggatctatcccaccaacggctacacaaggtatgccgactccgtgaagggatgtttcaccatctctgccgacacctccaagaataccgcctacctgcagatgaattccctgagggccgaagacacagctgtgtactactgctccaggtggggcggagatggcttttacgccatggactactggggacagggaacactggtgaccgtttcctcc

SEQ ID NO: 36 - protein, 120 aa, synthetic construct
EVQLVESGGGLVQPGGSLRLSCAASGFNIKDTYIHWVRQAPGKGLEWVARIYPTNGYTRYADSVKGCFTISADTSKNTAYLQMNSLRAEDTAVYYCSRWGGDGFYAMDYWGQGTLVTVSS

SEQ ID NO: 37 - DNA, 360 bp, synthetic construct
  source 1..360: mol_type = other DNA
gaagtgcagctggtggaatccggaggaggactggtgcaacctggagggtccctgaggttgtcttgtgctgcctccggcttcaacatcaaggacacctacatccactgggtgaggcaagctcctggcaaaggactggaatgggtggctaggatctatcccaccaacggctacacaaggtatgccgactccgtgaagggaaggttctgtatctctgccgacacctccaagaataccgcctacctgcagatgaattccctgagggccgaagacacagctgtgtactactgctccaggtggggcggagatggcttttacgccatggactactggggacagggaacactggtgaccgtttcctcc

SEQ ID NO: 38 - protein, 120 aa, synthetic construct
EVQLVESGGGLVQPGGSLRLSCAASGFNIKDTYIHWVRQAPGKGLEWVARIYPTNGYTRYADSVKGRFCISADTSKNTAYLQMNSLRAEDTAVYYCSRWGGDGFYAMDYWGQGTLVTVSS

SEQ ID NO: 39 - DNA, 360 bp, synthetic construct
  source 1..360: mol_type = other DNA
gaagtgcagctggtggaatccggaggaggactggtgcaacctggagggtccctgaggttgtcttgtgctgcctccggcttcaacatcaaggacacctacatccactgggtgaggcaagctcctggcaaaggactggaatgggtggctaggatctatcccaccaacggctacacaaggtatgccgactccgtgaagggaaggttcaccatctctgccgacacctccaagaattgtgcctacctgcagatgaattccctgagggccgaagacacagctgtgtactactgctccaggtggggcggagatggcttttacgccatggactactggggacagggaacactggtgaccgtttcctcc

SEQ ID NO: 40 - protein, 120 aa, synthetic construct
EVQLVESGGGLVQPGGSLRLSCAASGFNIKDTYIHWVRQAPGKGLEWVARIYPTNGYTRYADSVKGRFTISADTSKNCAYLQMNSLRAEDTAVYYCSRWGGDGFYAMDYWGQGTLVTVSS

SEQ ID NO: 41 - DNA, 360 bp, synthetic construct
  source 1..360: mol_type = other DNA
gaagtgcagctggtggaatccggaggaggactggtgcaacctggagggtccctgaggttgtcttgtgctgcctccggcttcaacatcaaggacacctacatccactgggtgaggcaagctcctggcaaaggactggaatgggtggctaggatctatcccaccaacggctacacaaggtatgccgactccgtgaagggaaggttcaccatctctgccgacacctccaagaatacctgttacctgcagatgaattccctgagggccgaagacacagctgtgtactactgctccaggtggggcggagatggcttttacgccatggactactggggacagggaacactggtgaccgtttcctcc

SEQ ID NO: 42 - protein, 120 aa, synthetic construct
EVQLVESGGGLVQPGGSLRLSCAASGFNIKDTYIHWVRQAPGKGLEWVARIYPTNGYTRYADSVKGRFTISADTSKNTCYLQMNSLRAEDTAVYYCSRWGGDGFYAMDYWGQGTLVTVSS

SEQ ID NO: 43 - DNA, 360 bp, synthetic construct
  source 1..360: mol_type = other DNA
gaagtgcagctggtggaatccggaggaggactggtgcaacctggagggtccctgaggttgtcttgtgctgcctccggcttcaacatcaaggacacctacatccactgggtgaggcaagctcctggcaaaggactggaatgggtggctaggatctatcccaccaacggctacacaaggtatgccgactccgtgaagggaaggttcaccatctctgccgacacctccaagaataccgcctacctgcagatgaattccctgagggccgaagacacagctgtgtactactgctccaggtggggcggagatggcttttacgccatggactactggggacagggatgtctggtgaccgtttcctcc

SEQ ID NO: 44 - protein, 120 aa, synthetic construct
EVQLVESGGGLVQPGGSLRLSCAASGFNIKDTYIHWVRQAPGKGLEWVARIYPTNGYTRYADSVKGRFTISADTSKNTAYLQMNSLRAEDTAVYYCSRWGGDGFYAMDYWGQGCLVTVSS

SEQ ID NO: 45 - DNA, 321 bp, synthetic construct
  source 1..321: mol_type = other DNA
gatatccagatgacccagtccccttcttccctgtccgcttctgtgggagacaggtgtacaatcacctgtagggcctcccaggacgtgaatacagctgtggcctggtaccaacaaaagcccggcaaagctcccaaactgctgatttactccgcctccttcctgtattctggagtgccctccaggttttctgggtccaggtccggaacagacttcacactgaccatctcctccctgcagcctgaagacttcgccacctactactgccagcagcactataccaccccccctacatttggacaaggcaccaaggtggagattaag

SEQ ID NO: 46 - protein, 107 aa, synthetic construct
DIQMTQSPSSLSASVGDRCTITCRASQDVNTAVAWYQQKPGKAPKLLIYSASFLYSGVPSRFSGSRSGTDFTLTISSLQPEDFATYYCQQHYTTPPTFGQGTKVEIK

SEQ ID NO: 47 - DNA, 321 bp, synthetic construct
  source 1..321: mol_type = other DNA
gatatccagatgacccagtccccttcttccctgtccgcttctgtgggagacagggtgacaatcacctgtagggcctcccaggacgtgaatacagctgtggcctggtaccaacaaaagcccggcaaagcttgtaaactgctgatttactccgcctccttcctgtattctggagtgccctccaggttttctgggtccaggtccggaacagacttcacactgaccatctcctccctgcagcctgaagacttcgccacctactactgccagcagcactataccaccccccctacatttggacaaggcaccaaggtggagattaag

SEQ ID NO: 48 - protein, 107 aa, synthetic construct
DIQMTQSPSSLSASVGDRVTITCRASQDVNTAVAWYQQKPGKACKLLIYSASFLYSGVPSRFSGSRSGTDFTLTISSLQPEDFATYYCQQHYTTPPTFGQGTKVEIK

SEQ ID NO: 49 - DNA, 321 bp, synthetic construct
  source 1..321: mol_type = other DNA
gatatccagatgacccagtccccttcttccctgtccgcttctgtgggagacagggtgacaatcacctgtagggcctcccaggacgtgaatacagctgtggcctggtaccaacaaaagcccggcaaagctcccaaatgtctgatttactccgcctccttcctgtattctggagtgccctccaggttttctgggtccaggtccggaacagacttcacactgaccatctcctccctgcagcctgaagacttcgccacctactactgccagcagcactataccaccccccctacatttggacaaggcaccaaggtggagattaag

SEQ ID NO: 50 - protein, 107 aa, synthetic construct
DIQMTQSPSSLSASVGDRVTITCRASQDVNTAVAWYQQKPGKAPKCLIYSASFLYSGVPSRFSGSRSGTDFTLTISSLQPEDFATYYCQQHYTTPPTFGQGTKVEIK

SEQ ID NO: 51 - DNA, 321 bp, synthetic construct
  source 1..321: mol_type = other DNA
gatatccagatgacccagtccccttcttccctgtccgcttctgtgggagacagggtgacaatcacctgtagggcctcccaggacgtgaatacagctgtggcctggtaccaacaaaagcccggcaaagctcccaaactgctgatttactccgcctccttcctgtattctggagtgccctccaggtgttctgggtccaggtccggaacagacttcacactgaccatctcctccctgcagcctgaagacttcgccacctactactgccagcagcactataccaccccccctacatttggacaaggcaccaaggtggagattaag

SEQ ID NO: 52 - protein, 107 aa, synthetic construct
DIQMTQSPSSLSASVGDRVTITCRASQDVNTAVAWYQQKPGKAPKLLIYSASFLYSGVPSRCSGSRSGTDFTLTISSLQPEDFATYYCQQHYTTPPTFGQGTKVEIK

SEQ ID NO: 53 - DNA, 321 bp, synthetic construct
  source 1..321: mol_type = other DNA
gatatccagatgacccagtccccttcttccctgtccgcttctgtgggagacagggtgacaatcacctgtagggcctcccaggacgtgaatacagctgtggcctggtaccaacaaaagcccggcaaagctcccaaactgctgatttactccgcctccttcctgtattctggagtgccctccaggttttctgggtccaggtccggaacagacttcacactgaccatctcctcctgtcagcctgaagacttcgccacctactactgccagcagcactataccaccccccctacatttggacaaggcaccaaggtggagattaag

SEQ ID NO: 54 - protein, 107 aa, synthetic construct
DIQMTQSPSSLSASVGDRVTITCRASQDVNTAVAWYQQKPGKAPKLLIYSASFLYSGVPSRFSGSRSGTDFTLTISSCQPEDFATYYCQQHYTTPPTFGQGTKVEIK

SEQ ID NO: 55 - DNA, 321 bp, synthetic construct
  source 1..321: mol_type = other DNA
gatatccagatgacccagtccccttcttccctgtccgcttctgtgggagacagggtgacaatcacctgtagggcctcccaggacgtgaatacagctgtggcctggtaccaacaaaagcccggcaaagctcccaaactgctgatttactccgcctccttcctgtattctggagtgccctccaggttttctgggtccaggtccggaacagacttcacactgaccatctcctccctgcagcctgaagacttcgccacctactgttgccagcagcactataccaccccccctacatttggacaaggcaccaaggtggagattaag

SEQ ID NO: 56 - protein, 107 aa, synthetic construct
DIQMTQSPSSLSASVGDRVTITCRASQDVNTAVAWYQQKPGKAPKLLIYSASFLYSGVPSRFSGSRSGTDFTLTISSLQPEDFATYCCQQHYTTPPTFGQGTKVEIK

SEQ ID NO: 57 - DNA, 360 bp, synthetic construct
  source 1..360: mol_type = other DNA
gaagtgcagctggtggaatccggaggaggactgtgtcaacctggagggtccctgaggttgtcttgtgctgcctccggcttcaacatcaaggacacctacatctgttgggtgaggcaagctcctggcaaaggactggaatgggtggctaggatctatcccaccaacggctacacaaggtatgccgactccgtgaagggaaggttcaccatctctgccgacacctccaagaataccgcctacctgcagatgaattccctgagggccgaagacacagctgtgtactactgctccaggtggggcggagatggcttttacgccatggactactggggacagggaacactggtgaccgtttcctcc

SEQ ID NO: 58 - protein, 120 aa, synthetic construct
EVQLVESGGGLCQPGGSLRLSCAASGFNIKDTYICWVRQAPGKGLEWVARIYPTNGYTRYADSVKGRFTISADTSKNTAYLQMNSLRAEDTAVYYCSRWGGDGFYAMDYWGQGTLVTVSS

SEQ ID NO: 59 - DNA, 360 bp, synthetic construct
  source 1..360: mol_type = other DNA
gaagtgcagctggtggaatccggaggaggactgtgtcaacctggagggtccctgaggttgtcttgtgctgcctccggcttcaacatcaaggacacctacatccactgggtgaggcaagctcctggcaaaggactggaatgggtggctaggatctatcccaccaacggctacacaaggtattgtgactccgtgaagggaaggttcaccatctctgccgacacctccaagaataccgcctacctgcagatgaattccctgagggccgaagacacagctgtgtactactgctccaggtggggcggagatggcttttacgccatggactactggggacagggaacactggtgaccgtttcctcc

SEQ ID NO: 60 - protein, 120 aa, synthetic construct
EVQLVESGGGLCQPGGSLRLSCAASGFNIKDTYIHWVRQAPGKGLEWVARIYPTNGYTRYCDSVKGRFTISADTSKNTAYLQMNSLRAEDTAVYYCSRWGGDGFYAMDYWGQGTLVTVSS

SEQ ID NO: 61 - DNA, 360 bp, synthetic construct
  source 1..360: mol_type = other DNA
gaagtgcagctggtggaatccggaggaggactggtgcaacctggagggtccctgaggttgtcttgtgctgcctccggcttcaacatcaaggacacctacatctgttgggtgaggcaagctcctggcaaaggactggaatgggtggctaggatctatcccaccaacggctacacaaggtattgtgactccgtgaagggaaggttcaccatctctgccgacacctccaagaataccgcctacctgcagatgaattccctgagggccgaagacacagctgtgtactactgctccaggtggggcggagatggcttttacgccatggactactggggacagggaacactggtgaccgtttcctcc

SEQ ID NO: 62 - protein, 120 aa, synthetic construct
EVQLVESGGGLVQPGGSLRLSCAASGFNIKDTYICWVRQAPGKGLEWVARIYPTNGYTRYCDSVKGRFTISADTSKNTAYLQMNSLRAEDTAVYYCSRWGGDGFYAMDYWGQGTLVTVSS

SEQ ID NO: 63 - DNA, 360 bp, synthetic construct
  source 1..360: mol_type = other DNA
gaagtgcagctggtggaatccggaggaggactggtgcaacctggagggtccctgaggttgtcttgtgctgcctccggcttcaacatcaaggacacctacatccactgggtgaggcaagctcctggcaaaggactggaatgggtggctaggtgttatcccaccaacggctacacaaggtattgtgactccgtgaagggaaggttcaccatctctgccgacacctccaagaataccgcctacctgcagatgaattccctgagggccgaagacacagctgtgtactactgctccaggtggggcggagatggcttttacgccatggactactggggacagggaacactggtgaccgtttcctcc

SEQ ID NO: 64 - protein, 120 aa, synthetic construct
EVQLVESGGGLVQPGGSLRLSCAASGFNIKDTYIHWVRQAPGKGLEWVARCYPTNGYTRYCDSVKGRFTISADTSKNTAYLQMNSLRAEDTAVYYCSRWGGDGFYAMDYWGQGTLVTVSS

SEQ ID NO: 65 - DNA, 321 bp, synthetic construct
  source 1..321: mol_type = other DNA
gatatccagatgacccagtccccttcttccctgtccgcttctgtgggagacagggtgacatgtacctgtagggcctcccaggacgtgaatacagctgtggcctggtaccaacaaaagcccggcaaagctcccaaactgtgtatttactccgcctccttcctgtattctggagtgccctccaggttttctgggtccaggtccggaacagacttcacactgaccatctcctccctgcagcctgaagacttcgccacctactactgccagcagcactataccaccccccctacatttggacaaggcaccaaggtggagattaag

SEQ ID NO: 66 - protein, 107 aa, synthetic construct
DIQMTQSPSSLSASVGDRVTCTCRASQDVNTAVAWYQQKPGKAPKLCIYSASFLYSGVPSRFSGSRSGTDFTLTISSLQPEDFATYYCQQHYTTPPTFGQGTKVEIK

SEQ ID NO: 67 - DNA, 321 bp, synthetic construct
  source 1..321: mol_type = other DNA
gatatccagatgacccagtccccttcttccctgtccgcttctgtgggagacagggtgacatgtacctgtagggcctcccaggacgtgaatacagctgtggcctggtaccaacaaaagcccggcaaagctcccaaactgctgtgttactccgcctccttcctgtattctggagtgccctccaggttttctgggtccaggtccggaacagacttcacactgaccatctcctccctgcagcctgaagacttcgccacctactactgccagcagcactataccaccccccctacatttggacaaggcaccaaggtggagattaag

SEQ ID NO: 68 - protein, 107 aa, synthetic construct
DIQMTQSPSSLSASVGDRVTCTCRASQDVNTAVAWYQQKPGKAPKLLCYSASFLYSGVPSRFSGSRSGTDFTLTISSLQPEDFATYYCQQHYTTPPTFGQGTKVEIK

SEQ ID NO: 69 - DNA, 321 bp, synthetic construct
  source 1..321: mol_type = other DNA
gatatccagatgacccagtccccttcttccctgtccgcttctgtgggagacagggtgacatgtacctgtagggcctcccaggacgtgaatacagctgtggcctggtaccaacaaaagcccggcaaagctcccaaactgctgatttactccgcctccttcctgtattctggagtgccctccaggttttctgggtccaggtccggaacagacttcacactgacctgttcctccctgcagcctgaagacttcgccacctactactgccagcagcactataccaccccccctacatttggacaaggcaccaaggtggagattaag

SEQ ID NO: 70 - protein, 107 aa, synthetic construct
DIQMTQSPSSLSASVGDRVTCTCRASQDVNTAVAWYQQKPGKAPKLLIYSASFLYSGVPSRFSGSRSGTDFTLTCSSLQPEDFATYYCQQHYTTPPTFGQGTKVEIK

SEQ ID NO: 71 - DNA, 321 bp, synthetic construct
  source 1..321: mol_type = other DNA
gatatccagatgacccagtccccttcttccctgtccgcttctgtgggagacagggtgacaatcacctgtagggcctcccaggacgtgaatacagctgtggcctggtaccaacaaaagcccggcaaagctcccaaatgtctgatttactccgcctccttcctgtattctggagtgccctccaggttttctgggtccaggtccggaacagacttcacactgaccatctcctccctgcagcctgaagacttcgccacctactgttgccagcagcactataccaccccccctacatttggacaaggcaccaaggtggagattaag

SEQ ID NO: 72 - protein, 107 aa, synthetic construct
DIQMTQSPSSLSASVGDRVTITCRASQDVNTAVAWYQQKPGKAPKCLIYSASFLYSGVPSRFSGSRSGTDFTLTISSLQPEDFATYCCQQHYTTPPTFGQGTKVEIK

SEQ ID NO: 73 - DNA, 357 bp, synthetic construct
  source 1..357: mol_type = other DNA
gaggtgcagctggtggagagcggcggcggcctggtgcagcccggcggcagcctgcgcctgagctgcgccgccagcggcttcaccttcaccgactacaccatggactgggtgcgccaggcccccggcaagggcctggagtgggtggccgacgtgaaccccaacagcggcggcagcatctacaaccagcgcttcaagggccgcttcaccctgagcgtggaccgcagcaagaacaccctgtacctgcagatgaacagcctgcgcgccgaggacaccgccgtgtactactgcgcccgcaacctgggccccagcttctacttcgactactggggccagggcaccctggtgaccgtgagcagc

SEQ ID NO: 74 - DNA, 321 bp, synthetic construct
  source 1..321: mol_type = other DNA
gacatccagatgacccagagccccagcagcctgagcgccagcgtgggcgaccgcgtgaccatcacctgcaaggccagccaggacgtgagcatcggcgtggcctggtaccagcagaagcccggcaaggcccccaagtgcctgatctacagcgccagctaccgctacaccggcgtgcccagccgcttcagcggcagcggcagcggcaccgacttcaccctgaccatcagcagcctgcagcccgaggacttcgccacctactactgccagcagtactacatctacccctacaccttcggccagggcaccaaggtggagatcaag

SEQ ID NO: 75 - protein, 119 aa, synthetic construct [sequence omitted]

SEQ ID NO: 76 - protein, 107 aa, synthetic construct
DIQMTQSPSSLSASVGDRVTITCKASQDVSIGVAWYQQKPGKAPKCLIYSASYRYTGVPSRFSGSGSGTDFTLTISSLQPEDFATYYCQQYYIYPYTFGQGTKVEIK

SEQ ID NO: 77 - DNA, 321 bp, synthetic construct
  source 1..321: mol_type = other DNA
gacatccagatgacccagagccccagcagcctgagcgccagcgtgggcgaccgcgtgaccatcacctgcaaggccagccaggacgtgagcatcggcgtggcctggtaccagcagaagcccggcaaggcccccaagctgctgatctacagcgccagctaccgctacaccggcgtgcccagccgcttcagcggcagcggcagcggcaccgacttcaccctgaccatcagcagcctgcagcccgaggacttcgccacctactgctgccagcagtactacatctacccctacaccttcggccagggcaccaaggtggagatcaag

SEQ ID NO: 78 - protein, 107 aa, synthetic construct
DIQMTQSPSSLSASVGDRVTITCKASQDVSIGVAWYQQKPGKAPKLLIYSASYRYTGVPSRFSGSGSGTDFTLTISSLQPEDFATYCCQQYYIYPYTFGQGTKVEIK

SEQ ID NO: 79 - DNA, 363 bp, synthetic construct
  source 1..363: mol_type = other DNA
caagtgcagctgcagcagcctggcgccgagctggtgaagcctggcgctagcgtgaagatgagctgcaaggctagcggctacaccttcacaagctacaacatgcactgggtgaagcagacccctggcagaggcctggagtggatcggcgccatctaccctggcaacggcgacacaagctacaatcagaagttcaagggcaaggccaccctgaccgccgacaagagcagcagcaccgcctacatgcagctgagcagcctgacaagcgaggacagcgccgtgtactactgcgctagaagcacctactacggcggcgactggtacttcaatgtgtggggagctggcaccaccgtcaccgtgagcgcc

SEQ ID NO: 80 - DNA, 318 bp, synthetic construct
  source 1..318: mol_type = other DNA
caaatcgtgctgagccaaagccctgccatcctgagcgctagccctggcgagaaggtgaccatgacctgcagagctagcagcagcgtgagctacatccactggtttcagcagaagcctggcagcagccctaagtgctggatctacgccacaagcaacctggctagcggcgtgcctgtgagattcagcggcagcggcagcggcacaagctacagcctgaccatcagcagagtggaggccgaggacgccgccacctactactgtcagcagtggacaagcaaccctcctaccttcggcggaggcaccaagctggagatcaag

SEQ ID NO: 81 - protein, 121 aa, synthetic construct [sequence omitted]

SEQ ID NO: 82 - protein, 106 aa, synthetic construct
QIVLSQSPAILSASPGEKVTMTCRASSSVSYIHWFQQKPGSSPKCWIYATSNLASGVPVRFSGSGSGTSYSLTISRVEAEDAATYYCQQWTSNPPTFGGGTKLEIK

SEQ ID NO: 83 - DNA, 357 bp, synthetic construct
  source 1..357: mol_type = other DNA
caagtgcagctgcagcagagcggcgccgagctggctagacctggcgctagcgtgaagatgagctgcaaggctagcggctacaccttcacaagatacaccatgcactgggtgaagcagagacctggccaaggcctggagtggatcggctacatcaaccctagcagaggctacaccaactacaatcagaagttcaaggacaaggccaccctgaccaccgacaagagcagcagcaccgcctacatgcagctgagcagcctgacaagcgaggacagcgccgtgtactactgcgctagatactacgacgaccactactgcctggactactggggccaaggcaccaccctgaccgtgagcagc

SEQ ID NO: 84 - DNA, 315 bp, synthetic construct
  source 1..315: mol_type = other DNA
caaatcgtgctgacacagagccctgccatcatgagcgctagccctggcgagaaggtgaccatgacctgcagcgctagcagcagcgtgagctacatgaactggtatcagcagaagagcggcacaagccctaagtgctggatctacgacacaagcaagctggctagcggcgtgcctgcccacttcagaggcagcggctccggcacatcctacagcctgaccatcagcggcatggaggccgaggacgccgccacctactactgtcagcagtggagcagcaaccctttcaccttcggcagcggcaccaagctggagatc

SEQ ID NO: 85 - protein, 119 aa, synthetic construct [sequence omitted]

SEQ ID NO: 86 - protein, 105 aa, synthetic construct
QIVLTQSPAIMSASPGEKVTMTCSASSSVSYMNWYQQKSGTSPKCWIYDTSKLASGVPAHFRGSGSGTSYSLTISGMEAEDAATYYCQQWSSNPFTFGSGTKLEI

SEQ ID NO: 87 - DNA, 348 bp, synthetic construct
  source 1..348: mol_type = other DNA
gaggtgcagctggtgcagagcggcggcggactggtgaagcctggcggcagcctgagactgagctgcgccgctagcggcttcaccttcagcagctacagcatgaactgggtgagacaagcccctggcaagggcctggagtgggtgagcagcatcagcagcagcagcagctacatctactacgccgacagcgtgaagggcagattcaccatcagcagagacaacgccaagaacagcctgtacctgcagatgaacagcctgagagccgaggacaccgccgtgtactactgcgctagagtgaccgacgccttcgacatctggggccaaggcacaatggtgacagtcagcagc

SEQ ID NO: 88 - DNA, 321 bp, synthetic construct
  source 1..321: mol_type = other DNA
gacattcagatgacacagagccctagcagcgtgagcgctagcatcggcgacagagtgaccatcacctgcagagctagccaaggcatcgacaactggctgggctggtatcagcagaagcctggcaaggcccctaagctgctgatctacgacgctagcaacctggacaccggcgtgcctagcagattcagcggcagcggcagcggcacctacttcaccctgaccatcagcagcctgcaagccgaggacttcgccgtgtactgctgtcagcaagccaaggccttccctcctaccttcggcggaggcaccaaggtggacatcaag

SEQ ID NO: 89 - protein, 116 aa, synthetic construct [sequence omitted]

SEQ ID NO: 90 - protein, 107 aa, synthetic construct
DIQMTQSPSSVSASIGDRVTITCRASQGIDNWLGWYQQKPGKAPKLLIYDASNLDTGVPSRFSGSGSGTYFTLTISSLQAEDFAVYCCQQAKAFPPTFGGGTKVDIK

SEQ ID NO: 91 - DNA, 321 bp, synthetic construct
  source 1..321: mol_type = other DNA
gacattcagatgacacagtcccctagcagcctgtccgcctccgtgggcgacagagtgaccatcacctgtaaggcctcccaagacgtgagcatcggcgtggcttggtaccaacaaaaacctggaaaggcccctaagctcctgatttacagcgcctcctatagatacaccggcgtgcctagcagattcagcggaagcggcagcggcaccgactttaccctgaccatcagcagcctgcagcctgaggatttcgctacctactattgccaacagtactacatctacccttacaccttcggccaaggcaccaaggtggagatcaag

SEQ ID NO: 92 - protein, 107 aa, synthetic construct [sequence omitted]

SEQ ID NO: 93 - DNA, 15 bp, synthetic construct
  source 1..15: mol_type = other DNA
ggaggaggaggcagc

SEQ ID NO: 94 - protein, 5 aa, synthetic construct
GGGGS

SEQ ID NO: 95 - protein, 106 aa, synthetic construct [sequence omitted]

SEQ ID NO: 96 - protein, 105 aa, synthetic construct
QIVLTQSPAIMSASPGEKVTMTCSASSSVSYMNWYQQKSGTSPKRWIYDTSKLASGVPAHFRGSGSGTSYSLTISGMEAEDAATYYCQQWSSNPFTFGSGTKLEI

SEQ ID NO: 97 - protein, 107 aa, synthetic construct [sequence omitted]

SEQ ID NO: 98 - DNA, 1350 bp, synthetic construct
  source 1..1350: mol_type = other DNA
gaagtgcaactggtggagtccggaggcggactggtccaacccggcggctctctgagactgagctgtgctgccagcggcttcaacatcaaggacacttacatccattgggtgaggcaagcccccggcaaaggactggaatgggtggctaggatctacccaactaacggctacactaggtatgccgacagcgtcaagggaaggttcactatctccgccgacacaagcaagaacactgcctatctgcagatgaactctctgagggctgaggacacagctgtgtattactgctctaggtggggcggagatggcttctacgctatggactactggggacaaggcacactcgtgacagtgagcagcgctagcactaaaggcccttccgtgttcccactcgcccctagctccaaaagcactagcggcggaacagctgctctgggctgtctcgtgaaggactatttcccagagccagtgactgtgagctggaatagcggcgctctgacaagcggagtgcacacttttccagccgtgctgcagagcagcggactgtattctctgtccagcgtcgtcactgtgcctagctcctctctgggcacacagacttacatctgtaacgtgaatcataagccaagcaacactaaggtcgacaagaaggtcgagccaaagagctgtgacaagacacacacatgcccaccatgtccagccccagagctcctcggaggacctagcgtgttcctcttccctcctaagccaaaggacactctcatgatctctaggacaccagaggtcacttgcgtggtggtcgatgtcagccacgaggacccagaggtgaagttcaattggtacgtggacggcgtggaggtgcataatgccaagacaaagcctagggaggagcagtacaacagcacttacagagtggtctccgtcctcacagtgctgcaccaagattggctcaacggcaaggagtacaagtgcaaggtgtccaacaaggccctcccagcccctatcgagaagactatctccaaggccaagggccagccaagagaacctcaagtgtacacactgcctccatctagggaggagatgacaaagaaccaagtgtctctgacatgtctggtgaaaggcttctacccaagcgacatcgccgtggagtgggaaagcaacggccagccagagaacaactacaagactacacctccagtgctggactccgacggcagcttcttcctctactccaagctcactgtggataagtctaggtggcagcaaggcaatgtgttcagctgttccgtgatgcacgaggctctgcacaaccactacactcagaagtctctgagcctctcccccggcaaa

SEQ ID NO: 99 - DNA, 642 bp, synthetic construct
  source 1..642: mol_type = other DNA
gacatccagatgacacagtccccttcctctctgagcgctagcgtcggcgatagggtgacaatcacttgtagggccagccaagatgtcaacacagccgtggcttggtaccagcagaagcccggcaaggcccctaagctgctcatctatagcgccagctttctgtacagcggcgtccctagcagattctccggaagcagatccggcactgacttcacactgactatcagcagcctccagccagaggatttcgccacatactactgccagcagcactacactactccacctactttcggccaaggcactaaggtggagattaagaggactgtcgctgccccaagcgtcttcatcttcccacctagcgatgaacagctcaagagcggcacagctagcgtcgtgtgtctgctgaacaacttctaccctagggaggccaaggtccagtggaaagtggataacgctctgcagagcggcaattcccaagagagcgtcacagagcaagatagcaaagacagcacttactctctgagcagcacactgactctgtccaaggccgactacgagaagcacaaggtctatgcttgtgaggtcactcaccaaggactgtccagcccagtcactaagagcttcaataggggcgagtgc

SEQ ID NO: 100 - protein, 450 aa, synthetic construct
EVQLVESGGGLVQPGGSLRLSCAASGFNIKDTYIHWVRQAPGKGLEWVARIYPTNGYTRYADSVKGRFTISADTSKNTAYLQMNSLRAEDTAVYYCSRWGGDGFYAMDYWGQGTLVTVSSASTKGPSVFPLAPSSKSTSGGTAALGCLVKDYFPEPVTVSWNSGALTSGVHTFPAVLQSSGLYSLSSVVTVPSSSLGTQTYICNVNHKPSNTKVDKKVEPKSCDKTHTCPPCPAPELLGGPSVFLFPPKPKDTLMISRTPEVTCVVVDVSHEDPEVKFNWYVDGVEVHNAKTKPREEQYNSTYRVVSVLTVLHQDWLNGKEYKCKVSNKALPAPIEKTISKAKGQPREPQVYTLPPSREEMTKNQVSLTCLVKGFYPSDIAVEWESNGQPENNYKTTPPVLDSDGSFFLYSKLTVDKSRWQQGNVFSCSVMHEALHNHYTQKSLSLSPGK

SEQ ID NO: 101 - protein, 214 aa, synthetic construct
DIQMTQSPSSLSASVGDRVTITCRASQDVNTAVAWYQQKPGKAPKLLIYSASFLYSGVPSRFSGSRSGTDFTLTISSLQPEDFATYYCQQHYTTPPTFGQGTKVEIKRTVAAPSVFIFPPSDEQLKSGTASVVCLLNNFYPREAKVQWKVDNALQSGNSQESVTEQDSKDSTYSLSSTLTLSKADYEKHKVYACEVTHQGLSSPVTKSFNRGEC

SEQ ID NO: 102 - DNA, 642 bp, synthetic construct
  source 1..642: mol_type = other DNA
gacatccagatgacacagtccccttcctctctgagcgctagcgtcggcgatagggtgacaatcacttgtagggccagccaagatgtcaacacagccgtggcttggtaccagcagaagcccggcaaggcccctaagtgtctcatctatagcgccagctttctgtacagcggcgtccctagcagattctccggaagcagatccggcactgacttcacactgactatcagcagcctccagccagaggatttcgccacatactactgccagcagcactacactactccacctactttcggccaaggcactaaggtggagattaagaggactgtcgctgccccaagcgtcttcatcttcccacctagcgatgaacagctcaagagcggcacagctagcgtcgtgtgtctgctgaacaacttctaccctagggaggccaaggtccagtggaaagtggataacgctctgcagagcggcaattcccaagagagcgtcacagagcaagatagcaaagacagcacttactctctgagcagcacactgactctgtccaaggccgactacgagaagcacaaggtctatgcttgtgaggtcactcaccaaggactgtccagcccagtcactaagagcttcaataggggcgagtgc

SEQ ID NO: 103 - protein, 214 aa, synthetic construct
DIQMTQSPSSLSASVGDRVTITCRASQDVNTAVAWYQQKPGKAPKCLIYSASFLYSGVPSRFSGSRSGTDFTLTISSLQPEDFATYYCQQHYTTPPTFGQGTKVEIKRTVAAPSVFIFPPSDEQLKSGTASVVCLLNNFYPREAKVQWKVDNALQSGNSQESVTEQDSKDSTYSLSSTLTLSKADYEKHKVYACEVTHQGLSSPVTKSFNRGEC

SEQ ID NO: 104 - DNA, 642 bp, synthetic construct
  source 1..642: mol_type = other DNA
gacatccagatgacacagtccccttcctctctgagcgctagcgtcggcgatagggtgacaatcacttgtagggccagccaagatgtcaacacagccgtggcttggtaccagcagaagcccggcaaggcccctaagctgctcatctatagcgccagctttctgtacagcggcgtccctagcagattctccggaagcagatccggcactgacttcacactgactatcagcagcctccagccagaggatttcgccacatactgttgccagcagcactacactactccacctactttcggccaaggcactaaggtggagattaagaggactgtcgctgccccaagcgtcttcatcttcccacctagcgatgaacagctcaagagcggcacagctagcgtcgtgtgtctgctgaacaacttctaccctagggaggccaaggtccagtggaaagtggataacgctctgcagagcggcaattcccaagagagcgtcacagagcaagatagcaaagacagcacttactctctgagcagcacactgactctgtccaaggccgactacgagaagcacaaggtctatgcttgtgaggtcactcaccaaggactgtccagcccagtcactaagagcttcaataggggcgagtgc

SEQ ID NO: 105 - protein, 214 aa, synthetic construct
DIQMTQSPSSLSASVGDRVTITCRASQDVNTAVAWYQQKPGKAPKLLIYSASFLYSGVPSRFSGSRSGTDFTLTISSLQPEDFATYCCQQHYTTPPTFGQGTKVEIKRTVAAPSVFIFPPSDEQLKSGTASVVCLLNNFYPREAKVQWKVDNALQSGNSQESVTEQDSKDSTYSLSSTLTLSKADYEKHKVYACEVTHQGLSSPVTKSFNRGEC

SEQ ID NO: 106 - DNA, 357 bp, synthetic construct
  source 1..357: mol_type = other DNA
caggtgcagctgaagcagagcggccccggcctggtgcagcccagccagagcctgagcatcacctgcaccgtgagcggcttcagcctgaccaactacggcgtgcactgggtgaggcagagccccggcaagggcctggagtggctgggcgtgatctggagcggcggcaacaccgactacaacacccccttcaccagcaggctgagcatcaacaaggacaacagcaagagccaggtgttcttcaagatgaacagcctgcagagcaacgacaccgccatctactactgcgccagggccctgacctactacgactacgagttcgcctactggggccagggcaccctggtgaccgtgagcgcc

SEQ ID NO: 107 - DNA, 321 bp, synthetic construct
  source 1..321: mol_type = other DNA
gacatcctgctgacccagagccccgtgatcctgagcgtgagccccggcgagagggtgagcttcagctgcagggccagccagagcatcggcaccaacatccactggtaccagcagaggaccaacggcagccccaggctgctgatcaagtacgccagcgagagcatcagcggcatccccagcaggttcagcggcagcggcagcggcaccgacttcaccctgagcatcaacagcgtggagagcgaggacatcgccgactactactgccagcagaacaacaactggcccaccaccttcggcgccggcaccaagctggagctgaag

SEQ ID NO: 108 - protein, 119 aa, synthetic construct
QVQLKQSGPGLVQPSQSLSITCTVSGFSLTNYGVHWVRQSPGKGLEWLGVIWSGGNTDYNTPFTSRLSINKDNSKSQVFFKMNSLQSNDTAIYYCARALTYYDYEFAYWGQGTLVTVSA

SEQ ID NO: 109 - protein, 107 aa, synthetic construct
DILLTQSPVILSVSPGERVSFSCRASQSIGTNIHWYQQRTNGSPRLLIKYASESISGIPSRFSGSGSGTDFTLSINSVESEDIADYYCQQNNNWPTTFGAGTKLELK

SEQ ID NO: 110 - DNA, 351 bp, synthetic construct
  source 1..351: mol_type = other DNA
caggtgcagctggtgcagagcggcgccgaggtgaagaagcccggcgccagcgtgaaggtgagctgcaaggccagcggctacaccttcaccagctacggcttcagctgggtgaggcaggcccccggccagggcctggagtggatgggctggatcagcgccagcaacggcaacacctactacgcccagaagctgcagggcagggtgaccatgaccaccgacaccagcaccagcaccgcctacatggagctgaggagcctgaggagcgacgacaccgccgtgtactactgcgccagggtgtacgccgactacgccgactactggggccagggcaccctggtgaccgtgagcagc

SEQ ID NO: 111 - DNA, 321 bp, synthetic construct
  source 1..321: mol_type = other DNA
gacatccagatgacccagagccccagcagcgtgagcgccagcgtgggcgacagggtgaccatcacctgcagggccagccagggcatcaacacctggctggcctggtaccagcagaagcccggcaaggcccccaagctgctgatctacgccgccagcagcctgaagagcggcgtgcccagcaggttcagcggcagcggcagcggcaccgacttcaccctgaccatcagcagcctgcagcccgaggacttcgccacctactactgccagcaggccaacagcttccccctgaccttcggcggcggcaccaaggtggagatcaag

SEQ ID NO: 112 - DNA, 54 bp, synthetic construct
  source 1..54: mol_type = other DNA
gtggagggcggcagcggcggcagcggcggcagcggcggcagcggcggcgtggac

SEQ ID NO: 113 - protein, 117 aa, synthetic construct
QVQLVQSGAEVKKPGASVKVSCKASGYTFTSYGFSWVRQAPGQGLEWMGWISASNGNTYYAQKLQGRVTMTTDTSTSTAYMELRSLRSDDTAVYYCARVYADYADYWGQGTLVTVSS

SEQ ID NO: 114 - protein, 107 aa, synthetic construct
DIQMTQSPSSVSASVGDRVTITCRASQGINTWLAWYQQKPGKAPKLLIYAASSLKSGVPSRFSGSGSGTDFTLTISSLQPEDFATYYCQQANSFPLTFGGGTKVEIK

SEQ ID NO: 115 - protein, 18 aa, synthetic construct
VEGGSGGSGGSGGSGGVD

SEQ ID NO: 116 - DNA, 321 bp, synthetic construct
  source 1..321: mol_type = other DNA
gacatcctgctgacccagagccccgtgatcctgagcgtgagccccggcgagagggtgagcttcagctgcagggccagccagagcatcggcaccaacatccactggtaccagcagaggaccaacggcagccccaggtgcctgatcaagtacgccagcgagagcatcagcggcatccccagcaggttcagcggcagcggcagcggcaccgacttcaccctgagcatcaacagcgtggagagcgaggacatcgccgactactactgccagcagaacaacaactggcccaccaccttcggcgccggcaccaagctggagctgaag

SEQ ID NO: 117 - protein, 107 aa, synthetic construct
DILLTQSPVILSVSPGERVSFSCRASQSIGTNIHWYQQRTNGSPRCLIKYASESISGIPSRFSGSGSGTDFTLSINSVESEDIADYYCQQNNNWPTTFGAGTKLELK

SEQ ID NO: 118 - DNA, 321 bp, synthetic construct
  source 1..321: mol_type = other DNA
gacatccagatgacccagagccccagcagcgtgagcgccagcgtgggcgacagggtgaccatcacctgcagggccagccagggcatcaacacctggctggcctggtaccagcagaagcccggcaaggcccccaagtgcctgatctacgccgccagcagcctgaagagcggcgtgcccagcaggttcagcggcagcggcagcggcaccgacttcaccctgaccatcagcagcctgcagcccgaggacttcgccacctactactgccagcaggccaacagcttccccctgaccttcggcggcggcaccaaggtggagatcaag

SEQ ID NO: 119 - protein, 107 aa, synthetic construct
DIQMTQSPSSVSASVGDRVTITCRASQGINTWLAWYQQKPGKAPKCLIYAASSLKSGVPSRFSGSGSGTDFTLTISSLQPEDFATYYCQQANSFPLTFGGGTKVEIK

SEQ ID NO: 120 - DNA, 321 bp, synthetic construct
  source 1..321: mol_type = other DNA
gacatccagatgacccagagccccagcagcgtgagcgccagcgtgggcgacagggtgaccatcacctgcagggccagccagggcatcaacacctggctggcctggtaccagcagaagcccggcaaggcccccaagctgctgatctacgccgccagcagcctgaagagcggcgtgcccagcaggttcagcggcagcggcagcggcaccgacttcaccctgaccatcagcagcctgcagcccgaggacttcgccacctactgctgccagcaggccaacagcttccccctgaccttcggcggcggcaccaaggtggagatcaag

SEQ ID NO: 121 - protein, 107 aa, synthetic construct
DIQMTQSPSSVSASVGDRVTITCRASQGINTWLAWYQQKPGKAPKLLIYAASSLKSGVPSRFSGSGSGTDFTLTISSLQPEDFATYCCQQANSFPLTFGGGTKVEIK

SEQ ID NO: 122 - DNA, 321 bp, synthetic construct
  source 1..321: mol_type = other DNA
gacatcctgctgacccagagccccgtgatcctgagcgtgagccccggcgagagggtgagcttcagctgcagggccagccagagcatcggcaccaacatccactggtaccagcagaggaccaacggcagccccaggctgctgatcaagtacgccagcgagagcatcagcggcatccccagcaggttcagcggcagcggcagcggcaccgacttcaccctgagcatcaacagcgtggagagcgaggacatcgccgactactgctgccagcagaacaacaactggcccaccaccttcggcgccggcaccaagctggagctgaag

SEQ ID NO: 123 - protein, 103 aa, synthetic construct
DILLTQSPVILSVSPGERVSFSCRASQSIGTNIHWYQQRTNGSPRLLIKYASESISGIPSRFSGSGSGTDFTLSINSVESEDIADYCCQQNNNWPTTFGAGTK

SEQ ID NO: 124 - DNA, 30 bp, synthetic construct
  source 1..30: mol_type = other DNA
ggcgggggcgggtccggcggcgggggcagc

SEQ ID NO: 125 - protein, 10 aa, synthetic construct
GGGGSGGGGS

SEQ ID NO: 126 - DNA, 60 bp, synthetic construct
  source 1..60: mol_type = other DNA
ggcgggggcgggtccggcggcgggggcagcgggggcggggggagcggcggggggggcagc

SEQ ID NO: 127 - protein, 25 aa, synthetic construct
GGGGSGGGGSGGGGSGGGGSGGGGS

SEQ ID NO: 128 - DNA, 375 bp, synthetic construct
  source 1..375: mol_type = other DNA
caagtgcagctggtggaatctggcggaggtgttgtgcagcctggcagaagcctgagactgtcctgcgccgctagcggcttcaccttcagcacctacggcatgcactgggtcagacaggcccctggaaaaggcctggagtgggtggccgtgatctgggacgacggctcttataagtactacggcgacagcgttaagggcaggttcaccatcagcagagataatagcaagaacaccctgtacctgcagatgaacagcctgcgggccgaggacactgccgtgtactactgtgccagagatggcatcacaatggtgcggggcgtgatgaaagactacttcgactactggggccagggcacactggtgacagtgtcctcc

SEQ ID NO: 129 - DNA, 321 bp, synthetic construct
  source 1..321: mol_type = other DNA
gctatccagctgacccagagcccaagcagcctgagcgcctctgtgggcgatagagtgaccattacatgcagagcctcccaggacatctctagtgctctggtgtggtaccagcaaaagcctggcaaggcccctaagtgcctgatctacgacgccagcagcctggaaagcggagtgcctagccggtttagcggcagcgagagcggcaccgacttcaccctgaccatcagctctctccagcccgaggattttgccacctattactgccagcagttcaacagctaccccctgacattcggcggaggaaccaaggtggaaatcaag

SEQ ID NO: 130 - protein, 125 aa, synthetic construct [sequence omitted]

SEQ ID NO: 131 - protein, 107 aa, synthetic construct
AIQLTQSPSSLSASVGDRVTITCRASQDISSALVWYQQKPGKAPKCLIYDASSLESGVPSRFSGSESGTDFTLTISSLQPEDFATYYCQQFNSYPLTFGGGTKVEIK

SEQ ID NO: 132 - DNA, 321 bp, synthetic construct
  source 1..321: mol_type = other DNA
gctatccagctgacccagagcccaagcagcctgagcgcctctgtgggcgatagagtgaccattacatgcagagcctcccaggacatctctagtgctctggtgtggtaccagcaaaagcctggcaaggcccctaagctgctgatctacgacgccagcagcctggaaagcggagtgcctagccggtttagcggcagcgagagcggcaccgacttcaccctgaccatcagctctctccagcccgaggattttgccacctattactgccagcagttcaacagctaccccctgacattcggcggaggaaccaaggtggaaatcaag

SEQ ID NO: 133 - protein, 107 aa, synthetic construct [sequence omitted]